European Patent Specification EP 3 928 101 B1, published October 9, 2024. Title: Methods of Determining Protein Stability. Applicant: Amgen Inc. The sequence listing filed with the application follows.

SEQUENCE LISTING (88 sequences)

SEQ ID NO: 1 - protein, 239 aa, Homo sapiens
MRLPAQLLGLLMLWVPGSSGDIVMTQTPLSSPVTLGQPASISCRSSQSLVHSDGNTYLNWLQQRPGQPPRLLIYKISNRFSGVPDRFTGSGAGTDFTLKISRVEAEDVGVYTCMQVTQFPLTFGQGTRLEIKRTVAAPSVFIFPPSDEQLKSGTASVVCLLNNFYPREAKVQWKVDNALQSGNSQESVTEQDSKDSTYSLSSTLTLSKADYEKHKVYACEVTHQGLSSPVTKSFNRGEC

SEQ ID NO: 2 - protein, 470 aa, Homo sapiens [sequence omitted]

SEQ ID NO: 3 - protein, 235 aa, Homo sapiens
METPAQLLFLLLLWLPDTTGEIVLTQSPGTLSLSPGDRATLSCRASQSVSSSYFAWYQQKPGQAPRLLIYGASSRATGIPDRFSGSGSGTDFTLTISRLEPEDFAVYYCQQYDRSPRTFGQGTKVEIKRTVAAPSVFIFPPSDEQLKSGTASVVCLLNNFYPREAKVQWKVDNALQSGNSQESVTEQDSKDSTYSLSSTLTLSKADYEKHKVYACEVTHQGLSSPVTKSFNRGEC

SEQ ID NO: 4 - protein, 463 aa, Homo sapiens
MDWTWRILFLVAAATGAHSQVQLVQSGAEVKKPGASVKVSCKSSGYTFTGYYMHWVRQAPGQGLEWMGWINPNSGGTNYAQKFKGRVTMTRDTSISTAYMELSRLRSDDTAVYYCARDKWLDGFDYWGQGTLVTVSSASTKGPSVFPLAPCSRSTSESTAALGCLVKDYFPEPVTVSWNSGALTSGVHTFPAVLQSSGLYSLSSVVTVPSSNFGTQTYTCNVDHKPSNTKVDKTVERKCCVECPPCPAPPVAGPSVFLFPPKPKDTLMISRTPEVTCVVVDVSHEDPEVQFNWYVDGVEVHNAKTKPREEQFNSTFRVVSVLTVVHQDWLNGKEYKCKVSNKGLPAPIEKTISKTKGQPREPQVYTLPPSREEMTKNQVSLTCLVKGFYPSDIAVEWESNGQPENNYKTTPPMLDSDGSFFLYSKLTVDKSRWQQGNVFSCSVMHEALHNHYTQKSLSLSPGK

SEQ ID NO: 5 - protein, 235 aa, Homo sapiens
MAWALLLLTLLTQDTGSWAQSVLTQSPSASGTPGQRVTISCSGSSSNIGSNYVYWYQQLPGAAPKLLILRNNQRPSGVPDRFSGSKSGTSASLTISGLRSEDEADYYCAAWDDSLSGWVFGGGTKLTVLGQPKANPTVTLFPPSSEELQANKATLVCLISDFYPGAVTVAWKADGSPVKAGVETTKPSKQSNNKYAASSYLSLTPEQWKSHRSYSCQVTHEGSTVEKTVAPTECS

SEQ ID NO: 6 - protein, 479 aa, Homo sapiens
MDMRVPAQLLGLLLLWLRGARCEVQLVESGGGLVKPGGSLRLSCAASGFTFSNAWMSWVRQAPGKGLEWVGRIKSKTDGGTTDYTAPVKGRFTISRDDSKNTLYLQMNSLKAEDTAVYYCTTDRTGYSISWSSYYYYYGMDVWGQGTTVTVSSASTKGPSVFPLAPCSRSTSESTAALGCLVKDYFPEPVTVSWNSGALTSGVHTFPAVLQSSGLYSLSSVVTVPSSNFGTQTYTCNVDHKPSNTKVDKTVERKCCVECPPCPAPPVAGPSVFLFPPKPKDTLMISRTPEVTCVVVDVSHEDPEVQFNWYVDGVEVHNAKTKPREEQFNSTFRVVSVLTVVHQDWLNGKEYKCKVSNKGLPAPIEKTISKTKGQPREPQVYTLPPSREEMTKNQVSLTCLVKGFYPSDIAVEWESNGQPENNYKTTPPMLDSDGSFFLYSKLTVDKSRWQQGNVFSCSVMHEALHNHYTQKSLSLSPGK

SEQ ID NO: 7 - protein, 235 aa, Homo sapiens
METPAQLLFLLLLWLPDTTGEIVLTQSPGTLSLSPGERATLSCRASQSVRGRYLAWYQQKPGQAPRLLIYGASSRATGIPDRFSGSGSGTDFTLTISRLEPEDFAVFYCQQYGSSPRTFGQGTKVEIKRTVAAPSVFIFPPSDEQLKSGTASVVCLLNNFYPREAKVQWKVDNALQSGNSQESVTEQDSKDSTYSLSSTLTLSKADYEKHKVYACEVTHQGLSSPVTKSFNRGEC

SEQ ID NO: 8 - protein, 467 aa, Homo sapiens
MEFGLSWLFLVAILKGVQCEVQLLESGGGLVQPGGSLRLSCAASGFTFSSYAMSWVRQAPGKGLEWVSGITGSGGSTYYADSVKGRFTISRDNSKNTLYLQMNSLRAEDTAVYYCAKDPGTTVIMSWFDPWGQGTLVTVSSASTKGPSVFPLAPCSRSTSESTAALGCLVKDYFPEPVTVSWNSGALTSGVHTFPAVLQSSGLYSLSSVVTVPSSNFGTQTYTCNVDHKPSNTKVDKTVERKCCVECPPCPAPPVAGPSVFLFPPKPKDTLMISRTPEVTCVVVDVSHEDPEVQFNWYVDGVEVHNAKTKPREEQFNSTFRVVSVLTVVHQDWLNGKEYKCKVSNKGLPAPIEKTISKTKGQPREPQVYTLPPSREEMTKNQVSLTCLVKGFYPSDIAVEWESNGQPENNYKTTPPMLDSDGSFFLYSKLTVDKSRWQQGNVFSCSVMHEALHNHYTQKSLSLSPGK

SEQ ID NO: 9 - protein, 242 aa, Homo sapiens
MDMRVPAQLLGLLLLWLRGARCDIVMTQTPLSLPVTPGEPASISCRSSQSLLNSVDGSTNLDWYLQKPGQSPQLLIYTLSYRASGVPDRFSGSGSGTDFTLKISRVEAEDVGVYYCMQRIEFPLTFGGGTKVEIKRTVAAPSVFIFPPSDEQLKSGTASVVCLLNNFYPREAKVQWKVDNALQSGNSQESVTEQDSKDSTYSLSSTLTLSKADYEKHKVYACEVTHQGLSSPVTKSFNRGEC

SEQ ID NO: 10 - protein, 465 aa, Homo sapiens
MELGLCWVFLVAILEGVQCEVQLVESGGGLVQPGGSLRLSCAASGFTFSSYSMNWVRQAPGKGLEWVSYISSSGSSIYYADSVKGRFTISRDNAKNSLYLQMNSLRDEDTAVYYCARERYYGDTPFDYWGQGTLVTVSSASTKGPSVFPLAPCSRSTSESTAALGCLVKDYFPEPVTVSWNSGALTSGVHTFPAVLQSSGLYSLSSVVTVPSSNFGTQTYTCNVDHKPSNTKVDKTVERKCCVECPPCPAPPVAGPSVFLFPPKPKDTLMISRTPEVTCVVVDVSHEDPEVQFNWYVDGVEVHNAKTKPREEQFNSTFRVVSVLTVVHQDWLNGKEYKCKVSNKGLPAPIEKTISKTKGQPREPQVYTLPPSREEMTKNQVSLTCLVKGFYPSDIAVEWESNGQPENNYKTTPPMLDSDGSFFLYSKLTVDKSRWQQGNVFSCSVMHEALHNHYTQKSLSLSPGK

SEQ ID NO: 11 - protein, 233 aa, Homo sapiens
MSPSQLIGFLLLWVPASRGEIVLTQSPDFQSVTPKEKVTITCRASQSIGSSLHWYQQKPDQSPKLLIKYASQSFSGVPSRFSGSGSGTDFTLTINSLEAEDAAAYYCHQSSSLPLTFGGGTKVEIKRTVAAPSVFIFPPSDEQLKSGTASVVCLLNNFYPREAKVQWKVDNALQSGNSQESVTEQDSKDSTYSLSSTLTLSKADYEKHKVYACEVTHQGLSSPVTKSFNRGEC

SEQ ID NO: 12 - protein, 463 aa, Homo sapiens
MGSTAILALLLAVLQGVCAEVQLMQSGAEVKKPGESLKISCKGSGYSFSFHWIAWVRQMPGKGLEWMGIIHPGASDTRYSPSFQGQVTISADNSNSATYLQWSSLKASDTAMYFCARQRELDYFDYWGQGTLVTVSSASTKGPSVFPLAPCSRSTSESTAALGCLVKDYFPEPVTVSWNSGALTSGVHTFPAVLQSSGLYSLSSVVTVPSSNFGTQTYTCNVDHKPSNTKVDKTVERKCCVECPPCPAPPVAGPSVFLFPPKPKDTLMISRTPEVTCVVVDVSHEDPEVQFNWYVDGVEVHNAKTKPREEQFNSTFRVVSVLTVVHQDWLNGKEYKCKVSNKGLPAPIEKTISKTKGQPREPQVYTLPPSREEMTKNQVSLTCLVKGFYPSDIAVEWESNGQPENNYKTTPPMLDSDGSFFLYSKLTVDKSRWQQGNVFSCSVMHEALHNHYTQKSLSLSPGK

SEQ ID NO: 13 - protein, 236 aa, Homo sapiens
MDMRVPAQLLGLLLLWLRGARCDIQMTQSPSSLSASVGDRVTITCKASQDINKYVAWYQQKPGKAPKLLIYYTSWLQPGVPSRFSGSGSGTDFTFTISSLQPEDIATYYCLQYDNLLYTFGQGTKLEIKRTVAAPSVFIFPPSDEQLKSGTASVVCLLNNFYPREAKVQWKVDNALQSGNSQESVTEQDSKDSTYSLSSTLTLSKADYEKHKVYACEVTHQGLSSPVTKSFNRGEC

SEQ ID NO: 14 - protein, 467 aa, Homo sapiens
MDMRVPAQLLGLLLLWLRGARCEVQLVESGGGLVQPGGSLRLSCAASGFTFSRYWMNWVRQAPGKGLEWVAQIRLKSDNYATHYAESVKGRFTISRDNAKNSLYLQMNSLRAEDTAVYYCTEGLDYWGQGTTVTVSSASTKGPSVFPLAPSSKSTSGGTAALGCLVKDYFPEPVTVSWNSGALTSGVHTFPAVLQSSGLYSLSSVVTVPSSSLGTQTYICNVNHKPSNTKVDKKVEPKSCDKTHTCPPCPAPELLGGPSVFLFPPKPKDTLMISRTPEVTCVVVDVSHEDPEVKFNWYVDGVEVHNAKTKPREEQYNSTYRVVSVLTVLHQDWLNGKEYKCKVSNKALPAPIEKTISKAKGQPREPQVYTLPPSREEMTKNQVSLTCLVKGFYPSDIAVEWESNGQPENNYKTTPPVLDSDGSFFLYSKLTVDKSRWQQGNVFSCSVMHEALHNHYTQKSLSLSPGK

SEQ ID NO: 15 - protein, 236 aa, Homo sapiens
MDMRVLAQLLGLLLLCFPGARCDIQMTQSPSSLSASVGDRVTITCRASQGISNWLAWYQQKPEKAPKSLIYAASSLQSGVPSRFSGSGSGTDFTLTISSLQPEDFATYYCQQYDSYPRTFGQGTKVEIKRTVAAPSVFIFPPSDEQLKSGTASVVCLLNNFYPREAKVQWKVDNALQSGNSQESVTEQDSKDSTYSLSSTLTLSKADYEKHKVYACEVTHQGLSSPVTKSFNRGEC

SEQ ID NO: 16 - protein, 466 aa, Homo sapiens
MELGLNWVFLVAILEGVHCEVQLVESGGGLVQPGGSLRLSCAASGFTFSSYWMSWVRQAPGKGLEWVAYIKQDGNEKYYVDSVKGRFTISRDNAKNSLYLQMNSLRAEDTAVYYCAREGILWFGDLPTFWGQGTLVTVSSASTKGPSVFPLAPCSRSTSESTAALGCLVKDYFPEPVTVSWNSGALTSGVHTFPAVLQSSGLYSLSSVVTVPSSNFGTQTYTCNVDHKPSNTKVDKTVERKCCVECPPCPAPPVAGPSVFLFPPKPKDTLMISRTPEVTCVVVDVSHEDPEVQFNWYVDGVEVHNAKTKPREEQFNSTFRVVSVLTVVHQDWLNGKEYKCKVSNKGLPAPIEKTISKTKGQPREPQVYTLPPSREEMTKNQVSLTCLVKGFYPSDIAVEWESNGQPENNYKTTPPMLDSDGSFFLYSKLTVDKSRWQQGNVFSCSVMHEALHNHYTQKSLSLSPGK

SEQ ID NO: 17 - protein, 241 aa, Homo sapiens
MDMRLPAQLLGLLMLWVPGSSGDVLMTQSPLSLPVTLGQPASISCRSSQSIVHSNGNTYLEWYLQRPGQSPKLLIYKVSNRFSGVPDRFSGSGSGTDFTLKISRVEAEDVGVYYCFQGSHVPLTFGAGTKLEIKRTVAAPSVFIFPPSDEQLKSGTASVVCLLNNFYPREAKVQWKVDNALQSGNSQESVTEQDSKDSTYSLSSTLTLSKADYEKHKVYACEVTHQGLSSPVTKSFNRGEC

SEQ ID NO: 18 - protein, 470 aa, Homo sapiens
MDTLCSTLLLLTIPSWVLSQVTLKESGPALVKPTQTLTLTCTFSGFSLRTSGMGVGWIRQPPGKALEWLAHIWWDDDKSYNPSLKSQLTISKDTSKNQVVLTMTNMDPVDTATYYCARRNYYYDDYFAYWGQGTLVTVSSASTKGPSVFPLAPSSKSTSGGTAALGCLVKDYFPEPVTVSWNSGALTSGVHTFPAVLQSSGLYSLSSVVTVPSSSLGTQTYICNVNHKPSNTKVDKKVEPKSCDKTHTCPPCPAPELLGGPSVFLFPPKPKDTLMISRTPEVTCVVVDVSHEDPEVKFNWYVDGVEVHNAKTKPREEQYNSTYRVVSVLTVLHQDWLNGKEYKCKVSNKALPAPIEKTISKAKGQPREPQVYTLPPSRDELTKNQVSLTCLVKGFYPSDIAVEWESNGQPENNYKTTPPVLDSDGSFFLYSKLTVDKSRWQQGNVFSCSVMHEALHNHYTQKSLSLSPGK

SEQ ID NO: 19 - protein, 235 aa, Homo sapiens
METPAQLLFLLLLWLPDTTGEIVLTQSPGTLSLSPGERATLSCRASQSVSSSYFAWYQQKPGQAPRLLIYGTSSRATGIPDRFSGSGSGTDFTLTVSRLEPEDFAVYYCQQYDRSPRTFGQGTKVEIKRTVAAPSVFIFPPSDEQLKSGTASVVCLLNNFYPREAKVQWKVDNALQSGNSQESVTEQDSKDSTYSLSSTLTLSKADYEKHKVYACEVTHQGLSSPVTKSFNRGEC

SEQ ID NO: 20 - protein, 463 aa, Homo sapiens
MDWTWRILFLVAAATGAHSQVQLVQSGAAVKKPGASVKVSCKASGYTFTGYYIHWVRQAPGQGLEWMGWINPNSGGTNYAQKFQGRVTMTRDTSISTASMELSRLRSDDTAVYFCARDRWLDAFDIWGQGTMVTVSSASTKGPSVFPLAPCSRSTSESTAALGCLVKDYFPEPVTVSWNSGALTSGVHTFPAVLQSSGLYSLSSVVTVPSSNFGTQTYTCNVDHKPSNTKVDKTVERKCCVECPPCPAPPVAGPSVFLFPPKPKDTLMISRTPEVTCVVVDVSHEDPEVQFNWYVDGVEVHNAKTKPREEQFNSTFRVVSVLTVVHQDWLNGKEYKCKVSNKGLPAPIEKTISKTKGQPREPQVYTLPPSREEMTKNQVSLTCLVKGFYPSDIAVEWESNGQPENNYKTTPPMLDSDGSFFLYSKLTVDKSRWQQGNVFSCSVMHEALHNHYTQKSLSLSPGK

SEQ ID NO: 21 - protein, 235 aa, Homo sapiens
METPAQLLFLLLLWLPDTTGEIVLTQSPGTLSLSPGERATLSCRASQSVSSGYLTWYQQKPGQAPRLLIYGASSRATGIPDRFSGSGSGTDFTLTISRLEPEDFAVYYCQQYGNSLSRFGQGTKLEIKRTVAAPSVFIFPPSDEQLKSGTASVVCLLNNFYPREAKVQWKVDNALQSGNSQESVTEQDSKDSTYSLSSTLTLSKADYEKHKVYACEVTHQGLSSPVTKSFNRGEC

SEQ ID NO: 22 - protein, 474 aa, Homo sapiens
MDMRVPAQLLGLLLLWLRGARCQVQLVESGGGVVQPGRSLRLSCAASGFTFSSYGMHWVRQAPGKGLEWVAVIWYDGSNKYYADSVKGRFIISRDKSKNTLYLQMNSLRAEDTAVYYCARAGGIAAAGLYYYYGMDVWGQGTTVTVSSASTKGPSVFPLAPCSRSTSESTAALGCLVKDYFPEPVTVSWNSGALTSGVHTFPAVLQSSGLYSLSSVVTVPSSNFGTQTYTCNVDHKPSNTKVDKTVERKCCVECPPCPAPPVAGPSVFLFPPKPKDTLMISRTPEVTCVVVDVSHEDPEVQFNWYVDGVEVHNAKTKPREEQFNSTFRVVSVLTVVHQDWLNGKEYKCKVSNKGLPAPIEKTISKTKGQPREPQVYTLPPSREEMTKNQVSLTCLVKGFYPSDIAVEWESNGQPENNYKTTPPMLDSDGSFFLYSKLTVDKSRWQQGNVFSCSVMHEALHNHYTQKSLSLSPGK

SEQ ID NO: 23 - protein, 236 aa, Homo sapiens
MDMRVPAQLLGLLLLWLRGARCSSELTQDPTVSVALGQTVKITCQGDSLRSFYASWYQQKPGQAPVLVFYGKNNRPSGIPDRFSGSSSGNTASLTITGAQAEDEADYYCNSRDSSVYHLVLGGGTKLTVLGQPKANPTVTLFPPSSEELQANKATLVCLISDFYPGAVTVAWKADGSPVKAGVETTKPSKQSNNKYAASSYLSLTPEQWKSHRSYSCQVTHEGSTVEKTVAPTECS

SEQ ID NO: 24 - protein, 478 aa, Homo sapiens
MDMRVPAQLLGLLLLWLRGARCQVQLVQSGAEVKKPGASVKVSCKASGYTFTGYYMHWVRQAPGQGLEWMGWINPNSGGTNYAQKFQGRVTMTRDTSISTAYMELSRLRSDDTAVYFCARDQMSIIMLRGVFPPYYYGMDVWGQGTTVTVSSASTKGPSVFPLAPCSRSTSESTAALGCLVKDYFPEPVTVSWNSGALTSGVHTFPAVLQSSGLYSLSSVVTVPSSNFGTQTYTCNVDHKPSNTKVDKTVERKCCVECPPCPAPPVAGPSVFLFPPKPKDTLMISRTPEVTCVVVDVSHEDPEVQFNWYVDGVEVHNAKTKPREEQFNSTFRVVSVLTVVHQDWLNGKEYKCKVSNKGLPAPIEKTISKTKGQPREPQVYTLPPSREEMTKNQVSLTCLVKGFYPSDIAVEWESNGQPENNYKTTPPMLDSDGSFFLYSKLTVDKSRWQQGNVFSCSVMHEALHNHYTQKSLSLSPGK

SEQ ID NO: 25 - protein, 241 aa, Homo sapiens
MDMRVPAQLLGLLLLWLRGARCDIVMTQSPLSLPVTPGEPASISCRSSQSLLHSNGYNYLDWYLQKPGQSPQLLIYLGSNRASGVPDRFSGSGSGTDFTLKISRVEAEDVGVYYCMQALQTPLTFGGGTKVEIKRTVAAPSVFIFPPSDEQLKSGTASVVCLLNNFYPREAKVQWKVDNALQSGNSQESVTEQDSKDSTYSLSSTLTLSKADYEKHKVYACEVTHQGLSSPVTKSFNRGEC

SEQ ID NO: 26 - protein, 475 aa, Homo sapiens
MDMRVPAQLLGLLLLWLRGARCEVQLVESGGGLVQPGGSLRLSCAASGFTFSSYWMSWVRQAPGKGLEWVASIKQDGSEKYYVDSVKGRFTISRDNARNSLYLQMNSLRAEDTAVYYCARDLVLMVYDIDYYYYGMDVWGQGTTVTVSSASTKGPSVFPLAPCSRSTSESTAALGCLVKDYFPEPVTVSWNSGALTSGVHTFPAVLQSSGLYSLSSVVTVPSSNFGTQTYTCNVDHKPSNTKVDKTVERKCCVECPPCPAPPVAGPSVFLFPPKPKDTLMISRTPEVTCVVVDVSHEDPEVQFNWYVDGVEVHNAKTKPREEQFNSTFRVVSVLTVVHQDWLNGKEYKCKVSNKGLPAPIEKTISKTKGQPREPQVYTLPPSREEMTKNQVSLTCLVKGFYPSDIAVEWESNGQPENNYKTTPPMLDSDGSFFLYSKLTVDKSRWQQGNVFSCSVMHEALHNHYTQKSLSLSPGK

SEQ ID NO: 27 - protein, 241 aa, Homo sapiens
MDMRVPAQLLGLLLLWLRGARCDIVMTQSPLSLPVTPGEPASISCRSSQSLLHSNGYNYLDWYLQKPGQSPQLLIYLGSNRASGVPDRFSGSGSGTHLTLKISRVEAEDVGVYYCMQTLQTPLTFGGGTKVEIKRTVAAPSVFIFPPSDEQLKSGTASVVCLLNNFYPREAKVQWKVDNALQSGNSQESVTEQDSKDSTYSLSSTLTLSKADYEKHKVYACEVTHQGLSSPVTKSFNRGEC

SEQ ID NO: 28 - protein, 475 aa, Homo sapiens
MDMRVPAQLLGLLLLWLRGARCEVQLVESGGGLVQPGGSLRLSCAASGFTFSNYWMSWVRQAPGKGLEWVASIKQDGSEKYYVDSVKGRFAISRDNAKNSLFLQMNSLRAEDTAVYYCARDLVLMVYDIDYYYYGMDVWGQGTTVTVSSASTKGPSVFPLAPCSRSTSESTAALGCLVKDYFPEPVTVSWNSGALTSGVHTFPAVLQSSGLYSLSSVVTVPSSNFGTQTYTCNVDHKPSNTKVDKTVERKCCVECPPCPAPPVAGPSVFLFPPKPKDTLMISRTPEVTCVVVDVSHEDPEVQFNWYVDGVEVHNAKTKPREEQFNSTFRVVSVLTVVHQDWLNGKEYKCKVSNKGLPAPIEKTISKTKGQPREPQVYTLPPSREEMTKNQVSLTCLVKGFYPSDIAVEWESNGQPENNYKTTPPMLDSDGSFFLYSKLTVDKSRWQQGNVFSCSVMHEALHNHYTQKSLSLSPGK

SEQ ID NO: 29 - protein, 235 aa, Homo sapiens
MTCSPLLLTLLIHCTGSWAQSVLTQPPSVSAAPGQKVTISCSGSSSNIGNNYVSWYQQLPGTAPKLLIYDNNKRPSGIPDRFSGSKSGTSTTLGITGLQTGDEADYYCGTWDSRLSAVVFGGGTKLTVLGQPKANPTVTLFPPSSEELQANKATLVCLISDFYPGAVTVAWKADGSPVKAGVETTKPSKQSNNKYAASSYLSLTPEQWKSHRSYSCQVTHEGSTVEKTVAPTECS

SEQ ID NO: 30 - protein, 475 aa, Homo sapiens
MEFGLSWVFLVALLRGVQCQVQLVESGGGVVQPGRSLRLSCAASGFTFSSFGMHWVRQAPGKGLEWVAVISFDGSIKYSVDSVKGRFTISRDNSKNTLFLQMNSLRAEDTAVYYCARDRLNYYDSSGYYHYKYYGMAVWGQGTTVTVSSASTKGPSVFPLAPCSRSTSESTAALGCLVKDYFPEPVTVSWNSGALTSGVHTFPAVLQSSGLYSLSSVVTVPSSNFGTQTYTCNVDHKPSNTKVDKTVERKCCVECPPCPAPPVAGPSVFLFPPKPKDTLMISRTPEVTCVVVDVSHEDPEVQFNWYVDGVEVHNAKTKPREEQFNSTFRVVSVLTVVHQDWLNGKEYKCKVSNKGLPAPIEKTISKTKGQPREPQVYTLPPSREEMTKNQVSLTCLVKGFYPSDIAVEWESNGQPENNYKTTPPMLDSDGSFFLYSKLTVDKSRWQQGNVFSCSVMHEALHNHYTQKSLSLSPGK

SEQ ID NO: 31 - protein, 234 aa, Homo sapiens
MDMRVPAQLLGLLLLWLRGARCYELTQPPSVSVSPGQTATITCSGDKLGERYASWYQQRPGQSPVLVIYQDIKRPSGIPERFSGSNSGNTATLTISGTQAMDEADYFCQAWYSSTNVLFGGGTKLTVLGQPKAAPSVTLFPPSSEELQANKATLVCLISDFYPGAVTVAWKADSSPVKAGVETTTPSKQSNNKYAASSYLSLTPEQWKSHRSYSCQVTHEGSTVEKTVAPTECS

SEQ ID NO: 32 - protein, 466 aa, Homo sapiens
MEFGLSWVFLVALLRGVQCQVQLVESGGGVVQPGRSLRLSCAASGFTFSSYGMHWVRQAPGKGLEWVAVIWYAESNKYYADSVKGRFTISRDNSKNTLYLQMNSLRAEDTAVYYCARAQEGIAPDAFDIWGQGTMVTVSSASTKGPSVFPLAPCSRSTSESTAALGCLVKDYFPEPVTVSWNSGALTSGVHTFPAVLQSSGLYSLSSVVTVPSSNFGTQTYTCNVDHKPSNTKVDKTVERKCCVECPPCPAPPVAGPSVFLFPPKPKDTLMISRTPEVTCVVVDVSHEDPEVQFNWYVDGVEVHNAKTKPREEQFNSTFRVVSVLTVVHQDWLNGKEYKCKVSNKGLPAPIEKTISKTKGQPREPQVYTLPPSREEMTKNQVSLTCLVKGFYPSDIAVEWESNGQPENNYKTTPPMLDSDGSFFLYSKLTVDKSRWQQGNVFSCSVMHEALHNHYTQKSLSLSPGK

SEQ ID NO: 33 - protein, 234 aa, Homo sapiens
MGSTAILGLLLAVLQGGRAEIVLTQSPGTLSLSPGERATLSCRASQSVSSSYLAWHQQKPGQAPRLLIYGASSRATGIPDRFSGSGSGTDFTLTISRLEPEDFAVYYCQQYGSSPWTFGQGTKVEIKRTVAAPSVFIFPPSDEQLKSGTASVVCLLNNFYPREAKVQWKVDNALQSGNSQESVTEQDSKDSTYSLSSTLTLSKADYEKHKVYACEVTHQGLSSPVTKSFNRGEC

SEQ ID NO: 34 - protein, 463 aa, Homo sapiens
MGSTAILGLLLAVLQGGRAEVQLLESGGGLVQPGGSLRLSCAASGFTFSTYVMSWVRQAPGKGLEWVSSISGSGLGSYYADSVKGRFTISRDNSKNTLYLQMNSLRAEDTAVYYCAKEAHRGPFDYWGQGTLVTVSSASTKGPSVFPLAPCSRSTSESTAALGCLVKDYFPEPVTVSWNSGALTSGVHTFPAVLQSSGLYSLSSVVTVPSSNFGTQTYTCNVDHKPSNTKVDKTVERKCCVECPPCPAPPVAGPSVFLFPPKPKDTLMISRTPEVTCVVVDVSHEDPEVQFNWYVDGVEVHNAKTKPREEQFNSTFRVVSVLTVVHQDWLNGKEYKCKVSNKGLPAPIEKTISKTKGQPREPQVYTLPPSREEMTKNQVSLTCLVKGFYPSDIAVEWESNGQPENNYKTTPPMLDSDGSFFLYSKLTVDKSRWQQGNVFSCSVMHEALHNHYTQKSLSLSPGK

SEQ ID NO: 35 - protein, 239 aa, Homo sapiens
MRLLAQLLGLLMLWVPGSSGDIVMTQTPLSSPVTLGQPASISCRSSQSLVHSDGNTYLSWLQQRPGQPPRLLIYKKFNRFSGVPDRFSGSGAGTDFTLKISRVEAEDVGVYYCMQATQIPLTFGPGTKVDIKRTVAAPSVFIFPPSDEQLKSGTASVVCLLNNFYPREAKVQWKVDNALQSGNSQESVTEQDSKDSTYSLSSTLTLSKADYEKHKVYACEVTHQGLSSPVTKSFNRGEC

SEQ ID NO: 36 - protein, 472 aa, Homo sapiens
MEFGLSWVFLVALLRGVQCQVQLVESGGGVVQPGRSLRLSCAASGFTFSFYGMHWVRQAPGKGLEWVAVIWYDGSNKYYADSVKGRFTISRDNSKNTLYLQMNSLRAEDTAVYYCARGGYDYVWGSYRRNSDFDYWGQGTLVTVSSASTKGPSVFPLAPCSRSTSESTAALGCLVKDYFPEPVTVSWNSGALTSGVHTFPAVLQSSGLYSLSSVVTVPSSNFGTQTYTCNVDHKPSNTKVDKTVERKCCVECPPCPAPPVAGPSVFLFPPKPKDTLMISRTPEVTCVVVDVSHEDPEVQFNWYVDGVEVHNAKTKPREEQFNSTFRVVSVLTVVHQDWLNGKEYKCKVSNKGLPAPIEKTISKTKGQPREPQVYTLPPSREEMTKNQVSLTCLVKGFYPSDIAVEWESNGQPENNYKTTPPMLDSDGSFFLYSKLTVDKSRWQQGNVFSCSVMHEALHNHYTQKSLSLSPGK

SEQ ID NO: 37 - protein, 235 aa, Homo sapiens
MEAPAQLLFLLLLWLPDTTGEIVMTQSPATLSVSPGERATLSCRASQSVDSNLAWYRQKPGQAPRLLIYGASTRATGIPARFSGSGSGTEFTLTISSLQSEDFAVYYCQQYINWPPITFGQGTRLEIKRTVAAPSVFIFPPSDEQLKSGTASVVCLLNNFYPREAKVQWKVDNALQSGNSQESVTEQDSKDSTYSLSSTLTLSKADYEKHKVYACEVTHQGLSSPVTKSFNRGEC

SEQ ID NO: 38 - protein, 465 aa, Homo sapiens
MKHLWFFLLLVAAPRWVLSQVQLQESGPGLVKPSETLSLTCTVSGGSISIYYWSWIRQPPGKGLEWIGYVYYSGSTNYNPSLKSRVTISVDTSKNQFSLKLNSVTAADTAVYYCARGGYDFWSGYFDYWGQGTLVTVSSASTKGPSVFPLAPCSRSTSESTAALGCLVKDYFPEPVTVSWNSGALTSGVHTFPAVLQSSGLYSLSSVVTVPSSNFGTQTYTCNVDHKPSNTKVDKTVERKCCVECPPCPAPPVAGPSVFLFPPKPKDTLMISRTPEVTCVVVDVSHEDPEVQFNWYVDGVEVHNAKTKPREEQFNSTFRVVSVLTVVHQDWLNGKEYKCKVSNKGLPAPIEKTISKTKGQPREPQVYTLPPSREEMTKNQVSLTCLVKGFYPSDIAVEWESNGQPENNYKTTPPMLDSDGSFFLYSKLTVDKSRWQQGNVFSCSVMHEALHNHYTQKSLSLSPGK

SEQ ID NO: 39 - protein, 240 aa, Homo sapiens
MVLQTQVFISLLLWISGAYGDIVLTQSPDSLAVSLGERATINCKSSQSILYSSSNENFLTWYQQKPGQPPKLLIYWASTRESGVPDRFSGSGSGTDFTLTISSLQPEDVAVYYCQQYFSVFRTFGQGTRVEIKRTVAAPSVFIFPPSDEQLKSGTASVVCLLNNFYPREAKVQWKVDNALQSGNSQESVTEQDSKDSTYSLSSTLTLSKADYEKHKVYACEVTHQGLSSPVTKSFNRGEC

SEQ ID NO: 40 - protein, 465 aa, Homo sapiens
MDWTWRILFLVAAATGAHSQVQLVQSGAEVKKPGASVKVSCKASGYTFTGYYIHWVRQAPGQGLEWMGWINPNSGGTNSAQKFRGRVTMTRDTSISTAYMELSRLRSDDTAVYYCAREGGYSYGYFDYWGQGTLVTVSSASTKGPSVFPLAPCSRSTSESTAALGCLVKDYFPEPVTVSWNSGALTSGVHTFPAVLQSSGLYSLSSVVTVPSSNFGTQTYTCNVDHKPSNTKVDKTVERKCCVECPPCPAPPVAGPSVFLFPPKPKDTLMISRTPEVTCVVVDVSHEDPEVQFNWYVDGVEVHNAKTKPREEQFNSTFRVVSVLTVVHQDWLNGKEYKCKVSNKGLPAPIEKTISKTKGQPREPQVYTLPPSREEMTKNQVSLTCLVKGFYPSDIAVEWESNGQPENNYKTTPPMLDSDGSFFLYSKLTVDKSRWQQGNVFSCSVMHEALHNHYTQKSLSLSPGK

SEQ ID NO: 41 - protein, 236 aa, Homo sapiens
MDMRVPAQLLGLLLLWFPGARCDIQMTQSPSSLSASVGDRVTITCRASQGIRNDLGWYQQKPGKAPKRLIYAASSLQSGVPSRFSGSGSGTEFTLTISSVQPEDFVTYYCLQHNSNPLTFGGGTKVEIKRTVAAPSVFIFPPSDEQLKSGTASVVCLLNNFYPREAKVQWKVDNALQSGNSQESVTEQDSKDSTYSLSSTLTLSKADYEKHKVYACEVTHQGLSSPVTKSFNRGEC

SEQ ID NO: 42 - protein, 473 aa, Homo sapiens
MEFGLSWVFLVALLRGVQCQVQLVESGGGVVQPGRSLRLSCAASGFTFSSYGMHWVRQAPGKGLEWVAVMWYDGSNKDYVDSVKGRFTISRDNSKNTLYLQMNRLRAEDTAVYYCAREKDHYDILTGYNYYYGLDVWGQGTTVTVSSASTKGPSVFPLAPCSRSTSESTAALGCLVKDYFPEPVTVSWNSGALTSGVHTFPAVLQSSGLYSLSSVVTVPSSNFGTQTYTCNVDHKPSNTKVDKTVERKCCVECPPCPAPPVAGPSVFLFPPKPKDTLMISRTPEVTCVVVDVSHEDPEVQFNWYVDGVEVHNAKTKPREEQFNSTFRVVSVLTVVHQDWLNGKEYKCKVSNKGLPAPIEKTISKTKGQPREPQVYTLPPSREEMTKNQVSLTCLVKGFYPSDIAVEWESNGQPENNYKTTPPMLDSDGSFFLYSKLTVDKSRWQQGNVFSCSVMHEALHNHYTQKSLSLSPGK

SEQ ID NO: 43 - protein, 235 aa, Homo sapiens
METPAQLLFLLLLWLPDTTGEIVLTQSPGTLSLSPGERATLSCRASQYISNTYLAWFQQKPGQAPRLLIYGAATRATGIPDRFSGSGSGTDFTFTISRLEPEDFAVYYCQQYGSSPWTFGQGTTVEIKRTVAAPSVFIFPPSDEQLKSGTASVVCLLNNFYPREAKVQWKVDNALQSGNSQESVTEQDSKDSTYSLSSTLTLSKADYEKHKVYACEVTHQGLSSPVTKSFNRGEC

SEQ ID NO: 44 - protein, 463 aa, Homo sapiens
MDWTWRILFLVAAATGAHSQVQLVQSGAEVKKPGASVKVSCKASGYTFTGYYMHWVRQAPGQGLEWMGWINPNSGGTNYAQRFRGRVTMTRDTSISTAYMELSRLRSDDTAVYYCARAPYDWTFDYWGQGTLVTVSSASTKGPSVFPLAPCSRSTSESTAALGCLVKDYFPEPVTVSWNSGALTSGVHTFPAVLQSSGLYSLSSVVTVPSSNFGTQTYTCNVDHKPSNTKVDKTVERKCCVECPPCPAPPVAGPSVFLFPPKPKDTLMISRTPEVTCVVVDVSHEDPEVQFNWYVDGVEVHNAKTKPREEQFNSTFRVVSVLTVVHQDWLNGKEYKCKVSNKGLPAPIEKTISKTKGQPREPQVYTLPPSREEMTKNQVSLTCLVKGFYPSDIAVEWESNGQPENNYKTTPPMLDSDGSFFLYSKLTVDKSRWQQGNVFSCSVMHEALHNHYTQKSLSLSPGK

SEQ ID NO: 45 - protein, 236 aa, Homo sapiens
MDMRVPAQLLGLLLLWLRGARCDIQMTQSPSSVSASVGDRVTITCRASQGISNWLAWYQQKPGTAPKLLIYAASSLQSGVPSRFSGSGSGTDFTLTISSLQPEDFATYYCQQANSFPFTFGPGTKVDIKRTVAAPSVFIFPPSDEQLKSGTASVVCLLNNFYPREAKVQWKVDNALQSGNSQESVTEQDSKDSTYSLSSTLTLSKADYEKHKVYACEVTHQGLSSPVTKSFNRGEC

SEQ ID NO: 46 - protein, 469 aa, Homo sapiens
MDMRVPAQLLGLLLLWLRGARCQVQLVQSGTEVKKPGASMKVSCKASGYTFTSYYMHWVRQAPGQGLEWMGIINPSGDSTSYAQKFQGRVTMTRDTSTNTVYMELSSLRSEDTAMYYCARDVEVRGISHFDYWGQGTLVTVSSASTKGPSVFPLAPCSRSTSESTAALGCLVKDYFPEPVTVSWNSGALTSGVHTFPAVLQSSGLYSLSSVVTVPSSNFGTQTYTCNVDHKPSNTKVDKTVERKCCVECPPCPAPPVAGPSVFLFPPKPKDTLMISRTPEVTCVVVDVSHEDPEVQFNWYVDGVEVHNAKTKPREEQFNSTFRVVSVLTVVHQDWLNGKEYKCKVSNKGLPAPIEKTISKTKGQPREPQVYTLPPSREEMTKNQVSLTCLVKGFYPSDIAVEWESNGQPENNYKTTPPMLDSDGSFFLYSKLTVDKSRWQQGNVFSCSVMHEALHNHYTQKSLSLSPGK

SEQ ID NO: 47 - protein, 238 aa, Homo sapiens
MGWSCIILFLVATATGVHSDIQLTQSPSSLSASVGDRVTMSCKSSQSVLYSANHKNYLAWYQQKPGKAPKLLIYWASTRESGVPSRFSGSGSGTDFTFTISSLQPEDIATYYCHQYLSSWTFGGGTKVQIKRTVAAPSVFIFPPSDEQLKSGTASVVCLLNNFYPREAKVQWKVDNALQSGNSQESVTEQDSKDSTYSLSSTLTLSKADYEKHKVYACEVTHQGLSSPVTKSFNRGEC

SEQ ID NO: 48 - protein, 465 aa, Homo sapiens
MGWSCIILFLVATATGVHSQVQLVQSGAEVKKPGSSVKVSCKASGYTFTSYWLHWVRQAPGQGLEWIGYINPRNDYTEYNQNFKDKATITADESTNTAYMELSSLRSEDTAFYFCARRDITTFYWGQGTTVTVSSASTKGPSVFPLAPSSKSTSGGTAALGCLVKDYFPEPVTVSWNSGALTSGVHTFPAVLQSSGLYSLSSVVTVPSSSLGTQTYICNVNHKPSNTKVDKRVEPKSCDKTHTCPPCPAPELLGGPSVFLFPPKPKDTLMISRTPEVTCVVVDVSHEDPEVKFNWYVDGVEVHNAKTKPREEQYNSTYRVVSVLTVLHQDWLNGKEYKCKVSNKALPAPIEKTISKAKGQPREPQVYTLPPSREEMTKNQVSLTCLVKGFYPSDIAVEWESNGQPENNYKTTPPVLDSDGSFFLYSKLTVDKSRWQQGNVFSCSVMHEALHNHYTQKSLSLSPGK

SEQ ID NO: 49 - protein, 235 aa, Homo sapiens
METPAQLLFLLLLWLPDTTGEIVLTQSPGTLSLSPGERATLSCRASQSVSSSYLAWYQQKPGQAPRLLIYGASSRATGIPDRFSGSGSGTDFTLTISRLEPEDFAVYYCQRSGGSSFTFGPGTKVDIKRTVAAPSVFIFPPSDEQLKSGTASVVCLLNNFYPREAKVQWKVDNALQSGNSQESVTEQDSKDSTYSLSSTLTLSKADYEKHKVYACEVTHQGLSSPVTKSFNRGEC

SEQ ID NO: 50 - protein, 466 aa, Homo sapiens
MGSTAILALLLAVLQGVCAEVQLVQSGAEVKKPGESLKISCKGSGYNFTSYWIGWVRQMPGKGLELMGIIYPGDSDTRYSPSFQGQVTISADKSISTAYLQWSSLKASDTAMYYCGSGSYFYFDLWGRGTLVTVSSASTKGPSVFPLAPSSKSTSGGTAALGCLVKDYFPEPVTVSWNSGALTSGVHTFPAVLQSSGLYSLSSVVTVPSSSLGTQTYICNVNHKPSNTKVDKKVEPKSCDKTHTCPPCPAPELLGGPSVFLFPPKPKDTLMISRTPEVTCVVVDVSHEDPEVKFNWYVDGVEVHNAKTKPREEQYNSTYRVVSVLTVLHQDWLNGKEYKCKVSNKALPAPIEKTISKAKGQPREPQVYTLPPSRDELTKNQVSLTCLVKGFYPSDIAVEWESNGQPENNYKTTPPVLDSDGSFFLYSKLTVDKSRWQQGNVFSCSVMHEALHNHYTQKSLSLSPGK

SEQ ID NO: 51 - protein, 241 aa, Homo sapiens
MDMRVPAQLLGLLLLWLRGARCDIVMTQSPLSLPVTPGEPASISCRSSQSLLHSHGYNYLDWYLQKPGQSPQLLIYLGSNRASGVPDRFSGSGSGTDFTLKISRVEAEDVGVYYCMQGTHWPPTFGQGTKLEIKRTVAAPSVFIFPPSDEQLKSGTASVVCLLNNFYPREAKVQWKVDNALQSGNSQESVTEQDSKDSTYSLSSTLTLSKADYEKHKVYACEVTHQGLSSPVTKSFNRGEC

SEQ ID NO: 52 - protein, 470 aa, Homo sapiens
MDMRVPAQLLGLLLLWLRGARCEVQLVQSGGGVVQPGRSLRLSCAASGFTFSSYGMHWVRQAPGKGLEWVSYISSSGSTIYYADSVKGRFTISRDNAKNSLYLQMNSLRAEDTAVYYCARDLLDYDLLTGYGYWGQGTLVTVSSASTKGPSVFPLAPCSRSTSESTAALGCLVKDYFPEPVTVSWNSGALTSGVHTFPAVLQSSGLYSLSSVVTVPSSNFGTQTYTCNVDHKPSNTKVDKTVERKCCVECPPCPAPPVAGPSVFLFPPKPKDTLMISRTPEVTCVVVDVSHEDPEVQFNWYVDGVEVHNAKTKPREEQFNSTFRVVSVLTVVHQDWLNGKEYKCKVSNKGLPAPIEKTISKTKGQPREPQVYTLPPSREEMTKNQVSLTCLVKGFYPSDIAVEWESNGQPENNYKTTPPMLDSDGSFFLYSKLTVDKSRWQQGNVFSCSVMHEALHNHYTQKSLSLSPGK

SEQ ID NO: 53 - protein, 235 aa, Homo sapiens
METPAQLLFLLLLWLPDTTGEIVLTQSPGTLSLSPGERATLSCRASQGISRSYLAWYQQKPGQAPSLLIYGASSRATGIPDRFSGSGSGTDFTLTISRLEPEDFAVYYCQQFGSSPWTFGQGTKVEIKRTVAAPSVFIFPPSDEQLKSGTASVVCLLNNFYPREAKVQWKVDNALQSGNSQESVTEQDSKDSTYSLSSTLTLSKADYEKHKVYACEVTHQGLSSPVTKSFNRGEC

SEQ ID NO: 54 - protein, 471 aa, Homo sapiens
MKHLWFFLLLVAAPRWVLSQVQLQESGPGLVKPSQTLSLTCTVSGGSISSGDYFWSWIRQLPGKGLEWIGHIHNSGTTYYNPSLKSRVTISVDTSKKQFSLRLSSVTAADTAVYYCARDRGGDYYYGMDVWGQGTTVTVSSASTKGPSVFPLAPSSKSTSGGTAALGCLVKDYFPEPVTVSWNSGALTSGVHTFPAVLQSSGLYSLSSVVTVPSSSLGTQTYICNVNHKPSNTKVDKRVEPKSCDKTHTCPPCPAPELLGGPSVFLFPPKPKDTLMISRTPEVTCVVVDVSHEDPEVKFNWYVDGVEVHNAKTKPREEQYNSTYRVVSVLTVLHQDWLNGKEYKCKVSNKALPAPIEKTISKAKGQPREPQVYTLPPSREEMTKNQVSLTCLVKGFYPSDIAVEWESNGQPENNYKTTPPVLDSDGSFFLYSKLTVDKSRWQQGNVFSCSVMHEALHNHYTQKSLSLSPGK

SEQ ID NO: 55 - protein, 236 aa, Homo sapiens
MDMRVPAQLLGLLLLWLSGARCDIQMTQSPSSLSASVGDRVTITCQASQDISNYLNWYQQKPGKAPKLLIYDASNLETGVPSRFSGSGSGTDFTFTISSLQPEDIATYFCQHFDHLPLAFGGGTKVEIKRTVAAPSVFIFPPSDEQLKSGTASVVCLLNNFYPREAKVQWKVDNALQSGNSQESVTEQDSKDSTYSLSSTLTLSKADYEKHKVYACEVTHQGLSSPVTKSFNRGEC

SEQ ID NO: 56 - protein, 464 aa, Homo sapiens
MKHLWFFLLLVAAPRWVLSQVQLQESGPGLVKPSETLSLTCTVSGGSVSSGDYYWTWIRQSPGKGLEWIGHIYYSGNTNYNPSLKSRLTISIDTSKTQFSLKLSSVTAADTAIYYCVRDRVTGAFDIWGQGTMVTVSSASTKGPSVFPLAPCSRSTSESTAALGCLVKDYFPEPVTVSWNSGALTSGVHTFPAVLQSSGLYSLSSVVTVPSSNFGTQTYTCNVDHKPSNTKVDKTVERKCCVECPPCPAPPVAGPSVFLFPPKPKDTLMISRTPEVTCVVVDVSHEDPEVQFNWYVDGVEVHNAKTKPREEQFNSTFRVVSVLTVVHQDWLNGKEYKCKVSNKGLPAPIEKTISKTKGQPREPQVYTLPPSREEMTKNQVSLTCLVKGFYPSDIAVEWESNGQPENNYKTTPPMLDSDGSFFLYSKLTVDKSRWQQGNVFSCSVMHEALHNHYTQKSLSLSPGK

SEQ ID NO: 57 - protein, 236 aa, Homo sapiens
METPAQLLFLLLLWLPDTASEIVLTQSPGTLSLSPGERATLSCRASQSVSNSYLAWYQQKPGQAPRLLIYGASSRAPGIPDRFSGSGSGTDFTLTISRLEPEDFAVYYCQQYDHSAGWTFGQGTKVEIKRTVAAPSVFIFPPSDEQLKSGTASVVCLLNNFYPREAKVQWKVDNALQSGNSQESVTEQDSKDSTYSLSSTLTLSKADYEKHKVYACEVTHQGLSSPVTKSFNRGEC

SEQ ID NO: 58 - protein, 460 aa, Homo sapiens
MGSTAILGLLLAVLQGVASEVQLVESGGGLVQPGGSLRLSCAASGFTFSRNAMFWVRQAPGKGLEWVSGIGTGGATSYADSVKGRFTISRDNAKNSLYLQMNSLRAEDTAVYYCARGRYYFPWWGQGTLVTVSSASTKGPSVFPLAPCSRSTSESTAALGCLVKDYFPEPVTVSWNSGALTSGVHTFPAVLQSSGLYSLSSVVTVPSSNFGTQTYTCNVDHKPSNTKVDKTVERKCCVECPPCPAPPVAGPSVFLFPPKPKDTLMISRTPEVTCVVVDVSHEDPEVQFNWYVDGVEVHNAKTKPREEQFNSTFRVVSVLTVVHQDWLNGKEYKCKVSNKGLPAPIEKTISKTKGQPREPQVYTLPPSREEMTKNQVSLTCLVKGFYPSDIAVEWESNGQPENNYKTTPPMLDSDGSFFLYSKLTVDKSRWQQGNVFSCSVMHEALHNHYTQKSLSLSPGK

SEQ ID NO: 59 - protein, 234 aa, Homo sapiens
METPAQLLFLLLLWLPDTTGEIVLTQSPGTLSLSPGERATLSCRASQSVSSSYLAWYQQKPGQAPRLLIYGASRRATGIPDRFSGSGSGTDFTLTISRLEPEDFAVYYCQRYGSSHTFGQGTKLEISRTVAAPSVFIFPPSDEQLKSGTASVVCLLNNFYPREAKVQWKVDNALQSGNSQESVTEQDSKDSTYSLSSTLTLSKADYEKHKVYACEVTHQGLSSPVTKSFNRGEC

SEQ ID NO: 60 - protein, 467 aa, Homo sapiens
MGSTAILALLLAVLQGVCAEVQLVQSGAEVKKPGESLKISCKVSGYFFTTYWIGWVRQMPGKGLEYMGIIYPGDSDTRYSPSFQGQVTISADKSISTAYLQWSSLKASDTAMYYCARGGNWNCFDYWGQGTLVTVSSASTKGPSVFPLAPSSKSTSGGTAALGCLVKDYFPEPVTVSWNSGALTSGVHTFPAVLQSSGLYSLSSVVTVPSSSLGTQTYICNVNHKPSNTKVDKRVEPKSCDKTHTCPPCPAPELLGGPSVFLFPPKPKDTLMISRTPEVTCVVVDVSHEDPEVKFNWYVDGVEVHNAKTKPREEQYNSTYRVVSVLTVLHQDWLNGKEYKCKVSNKALPAPIEKTISKAKGQPREPQVYTLPPSRDELTKNQVSLTCLVKGFYPSDIAVEWESNGQPENNYKTTPPVLDSDGSFFLYSKLTVDKSRWQQGNVFSCSVMHEALHNHYTQKSLSLSPGK

SEQ ID NO: 61 - protein, 241 aa, Homo sapiens
MDMRVPAQLLGLLLLWLRGARCDVVMTQSPLSLPVTPGEPASISCRSSQSLLHSNGYNYLDWYLQKPGQSPQLLIYLGSNRASGVPDRFSGSGSGTDFTLKISRVEAEDVGVYYCMQGTHWPLTFGQGTKVEIKRTVAAPSVFIFPPSDEQLKSGTASVVCLLNNFYPREAKVQWKVDNALQSGNSQESVTEQDSKDSTYSLSSTLTLSKADYEKHKVYACEVTHQGLSSPVTKSFNRGEC

SEQ ID NO: 62 - protein, 471 aa, Homo sapiens
MDMRVPAQLLGLLLLWLRGARCQVQLQESGPGLVKPSGTLSLTCAVSGGSISSSNWWSWVRQPPGKGLEWIGEIYHSGSTNYNPSLKSRVTISVDKSKNQFSLKLSSVTAADTAVYYCARWTGRTDAFDIWGQGTMVTVSSASTKGPSVFPLAPSSKSTSGGTAALGCLVKDYFPEPVTVSWNSGALTSGVHTFPAVLQSSGLYSLSSVVTVPSSSLGTQTYICNVNHKPSNTKVDKKVEPKSCDKTHTCPPCPAPELLGGPSVFLFPPKPKDTLMISRTPEVTCVVVDVSHEDPEVKFNWYVDGVEVHNAKTKPREEQYNSTYRVVSVLTVLHQDWLNGKEYKCKVSNKALPAPIEKTISKAKGQPREPQVYTLPPSRDELTKNQVSLTCLVKGFYPSDIAVEWESNGQPENNYKTTPPVLDSDGSFFLYSKLTVDKSRWQQGNVFSCSVMHEALHNHYTQKSLSLSPGK

SEQ ID NO: 63 - protein, 234 aa, Homo sapiens
MEAPAQLLFLLLLWLPDTTGEIVMTQSPATLSVSPGERATLSCRASQSVSSNLAWFQQKPGQAPRPLIYDASTRATGVPARFSGSGSGTDFTLTISSLQSEDFAVYYCQQYDNWPLTFGGGTKVEIKRTVAAPSVFIFPPSDEQLKSGTASVVCLLNNFYPREAKVQWKVDNALQSGNSQESVTEQDSKDSTYSLSSTLTLSKADYEKHKVYACEVTHQGLSSPVTKSFNRGEC

SEQ ID NO: 64 - protein, 461 aa, Homo sapiens
MEWTWRVLFLVAAATGAHSQVQLVQSGAEVKKPGASVKVSCKASGYTFTRYGISWVRQAPGQGLEWMGWISTYSGNTNYAQKLQGRVTMTTDTSTSTAYMELRSLRSDDTAVYYCARRQLYFDYWGQGTLVTVSSASTKGPSVFPLAPCSRSTSESTAALGCLVKDYFPEPVTVSWNSGALTSGVHTFPAVLQSSGLYSLSSVVTVPSSNFGTQTYTCNVDHKPSNTKVDKTVERKCCVECPPCPAPPVAGPSVFLFPPKPKDTLMISRTPEVTCVVVDVSHEDPEVQFNWYVDGVEVHNAKTKPREEQFNSTFRVVSVLTVVHQDWLNGKEYKCKVSNKGLPAPIEKTISKTKGQPREPQVYTLPPSREEMTKNQVSLTCLVKGFYPSDIAVEWESNGQPENNYKTTPPMLDSDGSFFLYSKLTVDKSRWQQGNVFSCSVMHEALHNHYTQKSLSLSPGK

SEQ ID NO: 65 - protein, 239 aa, Homo sapiens
MRLPAQLLGLLMLWIPGSSADIVMTQTPLSLSVTPGQPASISCKSGQSLLHSDGKTYLYWYLQKPGQPPQFLIYEVSNRFSRVPDRFSGSGSGTDFTLRISRVEAEDVGIYYCMQSIQLPWTFGQGTQVEIKRTVAAPSVFIFPPSDEQLKSGTASVVCLLNNFYPREAKVQWKVDNALQSGNSQESVTEQDSKDSTYSLSSTLTLSKADYEKHKVYACEVTHQGLSSPVTKSFNRGEC

SEQ ID NO: 66 - protein, 459 aa, Homo sapiens
MEFGLSWVFLVALLRGVQCQVQLVESGGGVVQPGRSLRLSCAASGFTFSGYGMHWVRQAPGKGLEWVAVISYDGNDKYYADSVKGRFTISRDNAKNTLYLQMNSLRAEDTAVYYCARELRVLWGQGTLVTVSSASTKGPSVFPLAPCSRSTSESTAALGCLVKDYFPEPVTVSWNSGALTSGVHTFPAVLQSSGLYSLSSVVTVPSSNFGTQTYTCNVDHKPSNTKVDKTVERKCCVECPPCPAPPVAGPSVFLFPPKPKDTLMISRTPEVTCVVVDVSHEDPEVQFNWYVDGVEVHNAKTKPREEQFNSTFRVVSVLTVVHQDWLNGKEYKCKVSNKGLPAPIEKTISKTKGQPREPQVYTLPPSREEMTKNQVSLTCLVKGFYPSDIAVEWESNGQPENNYKTTPPMLDSDGSFFLYSKLTVDKSRWQQGNVFSCSVMHEALHNHYTQKSLSLSPGK

SEQ ID NO: 67 - protein, 235 aa, Homo sapiens
MDMRVPAQLLGLLLLWLRGARCDIQMTQSPSSLSASVGDRVTITCRASQDISSYLNWYQQKPGKAPKLLIYSTSRLNSGVPSRFSGSGSGTDFTLTISSLQPEDFATYYCQQDIKHPTFGQGTKVEIKRTVAAPSVFIFPPSDEQLKSGTASVVCLLNNFYPREAKVQWKVDNALQSGNSQESVTEQDSKDSTYSLSSTLTLSKADYEKHKVYACEVTHQGLSSPVTKSFNRGEC

SEQ ID NO: 68 - protein, 465 aa, Homo sapiens
MDWTWRILFLVAAATGAHSEVQLVQSGAEVKKPGSSVKVSCKASGFTFTDYIMHWVRQAPGQGLEWMGYINPYNDDTEYNEKFKGRVTITADKSTSTAYMELSSLRSEDTAVYYCARSIYYYDAPFAYWGQGTLVTVSSASTKGPSVFPLAPCSRSTSESTAALGCLVKDYFPEPVTVSWNSGALTSGVHTFPAVLQSSGLYSLSSVVTVPSSNFGTQTYTCNVDHKPSNTKVDKTVERKCCVECPPCPAPPVAGPSVFLFPPKPKDTLMISRTPEVTCVVVDVSHEDPEVQFNWYVDGVEVHNAKTKPREEQFNSTFRVVSVLTVVHQDWLNGKEYKCKVSNKGLPAPIEKTISKTKGQPREPQVYTLPPSREEMTKNQVSLTCLVKGFYPSDIAVEWESNGQPENNYKTTPPMLDSDGSFFLYSKLTVDKSRWQQGNVFSCSVMHEALHNHYTQKSLSLSPGK

SEQ ID NO: 69 - protein, 233 aa, Homo sapiens
MGSTAILGLLLAVLQGGRASYVLTQPPSVSVAPGQTARITCGGNNLGSKSVHWYQQKPGQAPVLVVYDDSDRPSWIPERFSGSNSGNTATLTISRGEAGDEADYYCQVWDSSSDHVVFGGGTKLTVLGQPKAAPSVTLFPPSSEELQANKATLVCLISDFYPGAVTVAWKADSSPVKAGVETTTPSKQSNNKYAASSYLSLTPEQWKSHRSYSCQVTHEGSTVEKTVAPTECS

SEQ ID NO: 70 - protein, 467 aa, Homo sapiens
MGSTAILGLLLAVLQGGRAQMQLVESGGGVVQPGRSLRLSCAASGFTFRTYGMHWVRQAPGKGLEWVAVIWYDGSNKHYADSVKGRFTITRDNSKNTLNLQMNSLRAEDTAVYYCARAPQWELVHEAFDIWGQGTMVTVSSASTKGPSVFPLAPCSRSTSESTAALGCLVKDYFPEPVTVSWNSGALTSGVHTFPAVLQSSGLYSLSSVVTVPSSNFGTQTYTCNVDHKPSNTKVDKTVERKCCVECPPCPAPPVAGPSVFLFPPKPKDTLMISRTPEVTCVVVDVSHEDPEVQFNWYVDGVEVHNAKTKPREEQFNSTFRVVSVLTVVHQDWLNGKEYKCKVSNKGLPAPIEKTISKTKGQPREPQVYTLPPSREEMTKNQVSLTCLVKGFYPSDIAVEWESNGQPENNYKTTPPMLDSDGSFFLYSKLTVDKSRWQQGNVFSCSVMHEALHNHYTQKSLSLSPGK

SEQ ID NO: 71 - protein, 234 aa, Homo sapiens
MGVPTHLLGLLLLWITHAICDIRMTQSPASLSASLGETVNIECLASEDIYSDLAWYQQKPGKSPQLLIYNANSLQNGVPSRFSGSGSGTQYSLKINSLQSEDVATYFCQQYNNYPPTFGGGTKLELKRADAAPTVSIFPPSTEQLATGGASVVCLMNNFYPRDISVKWKIDGTERRDGVLDSVTDQDSKDSTYSMSSTLSLTKADYESHNLYTCEVVHKTSSSPVVKSFNRNEC

SEQ ID NO: 72 - protein, 465 aa, Homo sapiens
MDIRLSLAFLVLFIKGVQCEVQLVESGGGLVQPANSLKLSCAASGFTFSDYAMAWVRQSPKKGLEWVATIIYDGSSTYYRDSVKGRFTISRDNAKSTLYLQMDSLRSEDTATYYCATGLGIATDYFDYWGQGVLVTVSSAETTAPSVYPLAPGTALKSNSMVTLGCLVKGYFPEPVTVTWNSGALSSGVHTFPAVLQSGLYTLTSSVTVPSSTWPSQTVTCNVAHPASSTKVDKKIVPRNCGGDCKPCICTGSEVSSVFIFPPKPKDVLTITLTPKVTCVVVDISQDDPEVHFSWFVDDVEVHTAQTRPPEEQFNSTFRSVSELPILHQDWLNGRTFRCKVTSAAFPSPIEKTISKPEGRTQVPHVYTMSPTKEEMTQNEVSITCMVKGFYPPDIYVEWQMNGQPQENYKNTPPTMDTDGSYFLYSKLNVKKEKWQQGNTFTCSVLHEGLHNHHTEKSLSHSPGK

SEQ ID NO: 73 - protein, 237 aa, Homo sapiens
MDMRVPAQLLGLLLLWLRGARCESALTQPASVSGSPGQSITISCTGTSSDVGGYNSVSWYQQHPGKAPKLMIYEVSNRPSGVSNRFSGSKSGNTASLTISGLQAEDEADYYCNSYTSTSMVFGGGTKLTVLGQPKAAPSVTLFPPSSEELQANKATLVCLISDFYPGAVTVAWKADSSPVKAGVETTTPSKQSNNKYAASSYLSLTPEQWKSHRSYSCQVTHEGSTVEKTVAPTECS

SEQ ID NO: 74 - protein, 460 aa, Homo sapiens
MDWTWRILFLVAAATGVHSEVQLVQSGAEVKKPGASVKVSCKASGYTLTSYGISWVRQAPGQGLEWMGWVSFYNGNTNYAQKLQGRGTMTTDPSTSTAYMELRSLRSDDTAVYYCARGYGMDVWGQGTTVTVSSASTKGPSVFPLAPCSRSTSESTAALGCLVKDYFPEPVTVSWNSGALTSGVHTFPAVLQSSGLYSLSSVVTVPSSNFGTQTYTCNVDHKPSNTKVDKTVERKCCVECPPCPAPPVAGPSVFLFPPKPKDTLMISRTPEVTCVVVDVSHEDPEVQFNWYVDGVEVHNAKTKPREEQFNSTFRVVSVLTVVHQDWLNGKEYKCKVSNKGLPAPIEKTISKTKGQPREPQVYTLPPSREEMTKNQVSLTCLVKGFYPSDIAVEWESNGQPENNYKTTPPMLDSDGSFFLYSKLTVDKSRWQQGNVFSCSVMHEALHNHYTQKSLSLSPGK

SEQ ID NO: 75 - protein, 234 aa, Homo sapiens
METPAQLLFLLLLWLPDTTGEIVMTQSPATLSVSPGERATLSCRASQSVSSNLAWYQQKPGQAPRLLIYGAATRATGIPARVSGSGSGTEFTLTISSLQSEDFAVYYCQQYNNWPLTFGGGTKVEIKRTVAAPSVFIFPPSDEQLKSGTASVVCLLNNFYPREAKVQWKVDNALQSGNSQESVTEQDSKDSTYSLSSTLTLSKADYEKHKVYACEVTHQGLSSPVTKSFNRGEC

SEQ ID NO: 76 - protein, 472 aa, Homo sapiens
MDMRVPAQLLGLLLLWLRGARCQVQLVESGGGVVQPGRSLRLSCAASGFTFSNYGMHWVRQAPGEGLEWVAAIWFDASDKYYADAVKGRFTISRDNSKNTLYLQMNSLRAEDTAVYYCARDQAIFGVVPDYWGQGTLVTVSSASTKGPSVFPLAPSSKSTSGGTAALGCLVKDYFPEPVTVSWNSGALTSGVHTFPAVLQSSGLYSLSSVVTVPSSSLGTQTYICNVNHKPSNTKVDKKVEPKSCDKTHTCPPCPAPELLGGPSVFLFPPKPKDTLMISRTPEVTCVVVDVSHEDPEVKFNWYVDGVEVHNAKTKPCEEQYGSTYRCVSVLTVLHQDWLNGKEYKCKVSNKALPAPIEKTISKAKGQPREPQVYTLPPSREEMTKNQVSLTCLVKGFYPSDIAVEWESNGQPENNYKTTPPVLDSDGSFFLYSKLTVDKSRWQQGNVFSCSVMHEALHNHYTQKSLSLSPGK

SEQ ID NO: 77 - protein, 231 aa, Homo sapiens
MAWIPLFLGVLAYCTGSVASYEVTQAPSVSVSPGQTASITCSGDKLGDKYACWYQQKPGQSPVLVIYQDSKRPSGIPERFSGSNSGNTATLTISGTQAMDEADYYCQAWDSSTAVFGGGTKLTVLGQPKAAPSVTLFPPSSEELQANKATLVCLISDFYPGAVTVAWKADSSPVKAGVETTTPSKQSNNKYAASSYLSLTPEQWKSHRSYSCQVTHEGSTVEKTVAPTECS

SEQ ID NO: 78 - protein, 467 aa, Homo sapiens
MDWTWSILFLVAAATGAHSQVQLVQSGAEVKKPGASVKVSCKASGYTFTSYGLSWVRQAPGQGLEWMGWIIPYNGNTNSAQKLQGRVTMTTDTSTSTAYMELRSLRSDDTAVYFCARDRDYGVNYDAFDIWGQGTMVTVSSASTKGPSVFPLAPCSRSTSESTAALGCLVKDYFPEPVTVSWNSGALTSGVHTFPAVLQSSGLYSLSSVVTVPSSNFGTQTYTCNVDHKPSNTKVDKTVERKCCVECPPCPAPPVAGPSVFLFPPKPKDTLMISRTPEVTCVVVDVSHEDPEVQFNWYVDGVEVHNAKTKPREEQFNSTFRVVSVLTVVHQDWLNGKEYKCKVSNKGLPAPIEKTISKTKGQPREPQVYTLPPSREEMTKNQVSLTCLVKGFYPSDIAVEWESNGQPENNYKTTPPMLDSDGSFFLYSKLTVDKSRWQQGNVFSCSVMHEALHNHYTQKSLSLSPGK

SEQ ID NO: 79 - protein, 235 aa, Homo sapiens
MAWAPLLLTLLAHCTGSWANFMLTQPHSVSESPGKTVAISCTRNSGSIASNSVQWYQQRPGSSPTTVIFEDNQRPSGVPDRFSGSIDSSSNSASLTISGLKTEDEADYYCQSYDSNNWVFGGGTKLTVLGQPKANPTVTLFPPSSEELQANKATLVCLISDFYPGAVTVAWKADGSPVKAGVETTKPSKQSNNKYAASSYLSLTPEQWKSHRSYSCQVTHEGSTVEKTVAPTECS

SEQ ID NO: 80 - protein, 470 aa, Homo sapiens
MEFGLSWVFLVALLRGVQCQVQLVESGGGVVQPGRSLRLSCAASGFTFSSYVMHWVRQAPGKGLEWVAVIWYDGSNKYYADSVKGRFTISRDNSKNTLYLQMNSLRAEDTAVYYCAREGYDYGEDYYYYGMDVWGQGTTVTVSSASTKGPSVFPLAPCSRSTSESTAALGCLVKDYFPEPVTVSWNSGALTSGVHTFPAVLQSSGLYSLSSVVTVPSSNFGTQTYTCNVDHKPSNTKVDKTVERKCCVECPPCPAPPVAGPSVFLFPPKPKDTLMISRTPEVTCVVVDVSHEDPEVQFNWYVDGVEVHNAKTKPREEQFNSTFRVVSVLTVVHQDWLNGKEYKCKVSNKGLPAPIEKTISKTKGQPREPQVYTLPPSREEMTKNQVSLTCLVKGFYPSDIAVEWESNGQPENNYKTTPPMLDSDGSFFLYSKLTVDKSRWQQGNVFSCSVMHEALHNHYTQKSLSLSPGK

SEQ ID NO: 81 - protein, 236 aa, Homo sapiens
MDMRVPAQLLGLLLLWLRGARCDIQMTQSPSSLSASVGDRVTITCRASQDISNYLNWYQQKPGKAPKLLIYYTSRLLSGVPSRFSGSGSGTDFTLTISSLQPEDFATYYCQQGDTLPYTFGGGTKVEIKRTVAAPSVFIFPPSDEQLKSGTASVVCLLNNFYPREAKVQWKVDNALQSGNSQESVTEQDSKDSTYSLSSTLTLSKADYEKHKVYACEVTHQGLSSPVTKSFNRGEC

SEQ ID NO: 82 - protein, 468 aa, Homo sapiens
MDWTWRILFLVAAATGAHSEVQLVQSGAEVKKPGASVKVSCKASGYTFTDYNMHWVRQAPGQGLEWMGEINPNSGGAGYNQKFKGRVTMTTDTSTSTAYMELRSLRSDDTAVYYCARLGYDDIYDDWYFDVWGQGTTVTVSSASTKGPSVFPLAPCSRSTSESTAALGCLVKDYFPEPVTVSWNSGALTSGVHTFPAVLQSSGLYSLSSVVTVPSSNFGTQTYTCNVDHKPSNTKVDKTVERKCCVECPPCPAPPVAGPSVFLFPPKPKDTLMISRTPEVTCVVVDVSHEDPEVQFNWYVDGVEVHNAKTKPREEQFNSTFRVVSVLTVVHQDWLNGKEYKCKVSNKGLPAPIEKTISKTKGQPREPQVYTLPPSREEMTKNQVSLTCLVKGFYPSDIAVEWESNGQPENNYKTTPPMLDSDGSFFLYSKLTVDKSRWQQGNVFSCSVMHEALHNHYTQKSLSLSPGK

SEQ ID NO: 83 - protein, 240 aa, Homo sapiens
MVLQTQVFISLLLWISGAYGDIVMTQSPDSLAVSLGERATINCKSSQSVLDSSDNKNYLAWYQQKPGQPPKLLIYWASNRESGVPDRFSGSGSGTDFTLTISSLQAEDVAVYYCQQYYSDPFTFGPGTKVDIKRTVAAPSVFIFPPSDEQLKSGTASVVCLLNNFYPREAKVQWKVDNALQSGNSQESVTEQDSKDSTYSLSSTLTLSKADYEKHKVYACEVTHQGLSSPVTKSFNRGEC

SEQ ID NO: 84 - protein, 465 aa, Homo sapiens
MDWTWSILFLVAAPTGAHSQVQLVQSGAEVKKPGASVKVSCKASGYTFTSYGISWVRQAPGQGLEWMGWISAYNGNTNYAQKLQGRVTMTTDTSTSTAYMELRSLRSDDTAVYYCARESWFGEVFFDYWGQGTLVTVSSASTKGPSVFPLAPCSRSTSESTAALGCLVKDYFPEPVTVSWNSGALTSGVHTFPAVLQSSGLYSLSSVVTVPSSNFGTQTYTCNVDHKPSNTKVDKTVERKCCVECPPCPAPPVAGPSVFLFPPKPKDTLMISRTPEVTCVVVDVSHEDPEVQFNWYVDGVEVHNAKTKPREEQFNSTFRVVSVLTVVHQDWLNGKEYKCKVSNKGLPAPIEKTISKTKGQPREPQVYTLPPSREEMTKNQVSLTCLVKGFYPSDIAVEWESNGQPENNYKTTPPMLDSDGSFFLYSKLTVDKSRWQQGNVFSCSVMHEALHNHYTQKSLSLSPGK

SEQ ID NO: 85 - protein, 236 aa, Homo sapiens
MDMRVPAQLLGLLLLWLRGARCDIQMTQSPSSVSASVGDRVTITCRASQGISSWLAWYQQKPGKAPKLLIYGASNLESGVPSRFSGSGSGTDFTLTISSLQPEDFANYYCQQANSFPWTFGQGTKVEIKRTVAAPSVFIFPPSDEQLKSGTASVVCLLNNFYPREAKVQWKVDNALQSGNSQESVTEQDSKDSTYSLSSTLTLSKADYEKHKVYACEVTHQGLSSPVTKSFNRGEC

SEQ ID NO: 86 - protein, 466 aa, Homo sapiens
MDMRVPAQLLGLLLLWLRGARCQVQLVQSGAEVKKPGASVKVSCKVSGYTLSDLSIHWVRQAPGKGLEWMGGFDPQDGETIYAQKFQGRVTMTEDTSTDTAYMELSSLKSEDTAVYYCATGSSSSWFDPWGQGTLVTVSSASTKGPSVFPLAPCSRSTSESTAALGCLVKDYFPEPVTVSWNSGALTSGVHTFPAVLQSSGLYSLSSVVTVPSSNFGTQTYTCNVDHKPSNTKVDKTVERKCCVECPPCPAPPVAGPSVFLFPPKPKDTLMISRTPEVTCVVVDVSHEDPEVQFNWYVDGVEVHNAKTKPREEQFNSTFRVVSVLTVVHQDWLNGKEYKCKVSNKGLPAPIEKTISKTKGQPREPQVYTLPPSREEMTKNQVSLTCLVKGFYPSDIAVEWESNGQPENNYKTTPPMLDSDGSFFLYSKLTVDKSRWQQGNVFSCSVMHEALHNHYTQKSLSLSPGK

SEQ ID NO: 87 - protein, 472 aa, Homo Sapiens
MDMRVPAQLLGLLLLWLRGARCEVQLLESGGGLVQPGGSLRLSCAASGFTFSSYDMSWVRQAPGKGLEWVSLISGGGSQTYYAESVKGRFTISRDNSKNTLYLQMNSLRAEDTAVYFCASPSGHYFYAMDVWGQGTTVTVSSASTKGPSVFPLAPSSKSTSGGTAALGCLVKDYFPEPVTVSWNSGALTSGVHTFPAVLQSSGLYSLSSVVTVPSSSLGTQTYICNVNHKPSNTKVDKKVEPKSCDKTHTCPPCPAPELLGGPSVFLFPPKPKDTLMISRTPEVTCVVVDVSHEDPEVKFNWYVDGVEVHNAKTKPCEEQYGSTYRCVSVLTVLHQDWLNGKEYKCKVSNKALPAPIEKTISKAKGQPREPQVYTLPPSREEMTKNQVSLTCLVKGFYPSDIAVEWESNGQPENNYKTTPPVLDSDGSFFLYSKLTVDKSRWQQGNVFSCSVMHEALHNHYTQKSLSLSPGK

SEQ ID NO: 88 - protein, 236 aa, Homo Sapiens
MDMRVPAQLLGLLLLWLRGARCDIQMTQSPSSVSASVGDRVTITCRASQGISNWLAWYQQKPGKAPKLLIFAASSLQSGVPSRFSGSGSGTDFTLTISSLQPEDFATYYCQQAESFPHTFGGGTKVEIKRTVAAPSVFIFPPSDEQLKSGTASVVCLLNNFYPREAKVQWKVDNALQSGNSQESVTEQDSKDSTYSLSSTLTLSKADYEKHKVYACEVTHQGLSSPVTKSFNRGEC